European Patent Application EP 4 148 042 A1, published March 15, 2023. Title: Phenoxy-acetyl-thioureido-benzenesulfonamide derivatives, and their uses. Applicant: Centre National de la Recherche Scientifique Universite de Montpellier. The sequence listing filed with the application follows.

SEQUENCE LISTING (22 sequences)

SEQ ID NO: 1 - DNA, 29 bp, Artificial sequence
  oligonucleotide for amplification
ttgcggccgcgccaccatgagcgataacg

SEQ ID NO: 2 - DNA, 19 bp, Artificial sequence
  oligonucleotide for amplification
cgcctgagtagaatcggct

SEQ ID NO: 3 - DNA, 38 bp, Artificial sequence
  oligonucleotide for amplification
agccgattctactcaggcgggaggttctggtggttctg

SEQ ID NO: 4 - DNA, 29 bp, Artificial sequence
  oligonucleotide for amplification
gaggatcctcacttgtacagctcgtccat

SEQ ID NO: 5 - DNA, 15 bp, Artificial sequence
  oligonucleotide for amplification
ttgcggccgcgccac

SEQ ID NO: 6 - DNA, 25 bp, Artificial sequence
  oligonucleotide for amplification
gaggatcctcacttgtacagctcgt

SEQ ID NO: 7 - DNA, 21 bp, Artificial sequence
  oligonucleotide for amplification
ctgagtccgaatcaggtgcag

SEQ ID NO: 8 - DNA, 21 bp, Artificial sequence
  oligonucleotide for amplification
atccatggggagatgttctgg

SEQ ID NO: 9 - DNA, 20 bp, Artificial sequence
  oligonucleotide for amplification
cagcactcagactacgtgca

SEQ ID NO: 10 - DNA, 21 bp, Artificial sequence
  oligonucleotide for amplification
atccatggggagatgttctgg

SEQ ID NO: 11 - DNA, 21 bp, Artificial sequence
  oligonucleotide for amplification
tggccgggtctgctgagtccg

SEQ ID NO: 12 - DNA, 21 bp, Artificial sequence
  oligonucleotide for amplification
atccatggggagatgttctgg

SEQ ID NO: 13 - DNA, 20 bp, Artificial sequence
  oligonucleotide for amplification
gttctccagcgacaaggcta

SEQ ID NO: 14 - DNA, 20 bp, Artificial sequence
  oligonucleotide for amplification
atcctgcttgctgttgttgg

SEQ ID NO: 15 - DNA, 22 bp, Artificial sequence
  oligonucleotide for amplification
agaaccaggaaacggaaacaga

SEQ ID NO: 16 - DNA, 20 bp, Artificial sequence
  oligonucleotide for amplification
tctccttcatgcgctgcttt

SEQ ID NO: 17 - DNA, 25 bp, Artificial sequence
  oligonucleotide for amplification
tgttcaaccaattatcagcaaactc

SEQ ID NO: 18 - DNA, 24 bp, Artificial sequence
  oligonucleotide for amplification
ttctgctgtatcctcttcaccagt

SEQ ID NO: 19 - DNA, 18 bp, Artificial sequence
  oligonucleotide for amplification
gaaacggatgcctggtgg

SEQ ID NO: 20 - DNA, 18 bp, Artificial sequence
  oligonucleotide for amplification
gccccttcttcctgggtc

SEQ ID NO: 21 - DNA, 19 bp, Artificial sequence
  oligonucleotide for amplification
caagtgtgggtacgccacg

SEQ ID NO: 22 - DNA, 21 bp, Artificial sequence
  oligonucleotide for amplification
aaagaagctctccatccggtc